European Patent Application EP 4 628 097 A1, published October 8, 2025. Title: 包含结合VEGF和Ang2的双特异性结合分子的制剂以及其用途. Applicant: 信达生物制药（苏州）有限公司. The sequence listing filed with the application follows.

SEQUENCE LISTING (48 sequences)

SEQ ID NO: 1 - protein, 10 aa, synthetic construct
  REGION 1..10: note = Synthetic construct
GFNLDYYPIG

SEQ ID NO: 2 - protein, 16 aa, synthetic construct
  REGION 1..16: note = Synthetic construct
CISSVGSTNYADSVKG

SEQ ID NO: 3 - protein, 15 aa, synthetic construct
  REGION 1..15: note = Synthetic construct
DPLCSALILPPPFLS

SEQ ID NO: 4 - protein, 123 aa, synthetic construct
  REGION 1..123: note = Synthetic construct
QLQLVESGGGLVQPGGSLRLSCAASGFNLDYYPIGWFRQAPGKEREGVSCISSVGSTNYADSVKGRFTISRDNAKNTVYLQMNSLKPEDTAVYYCAADPLCSALILPPPFLSWGQGTQVTVSS

SEQ ID NO: 5 - protein, 123 aa, synthetic construct
  REGION 1..123: note = Synthetic construct
EVQLLESGGGLVQPGGSLRLSCAASGFNLDYYPIGWFRQAPGKGLEGVSCISSVGSTNYADSVKGRFTISRDNSKNTVYLQMNSLRAEDTAVYYCAADPLCSALILPPPFLSWGQGTQVTVSS

SEQ ID NO: 6 - protein, 10 aa, synthetic construct
  REGION 1..10: note = Synthetic construct
GSIFSINAMG

SEQ ID NO: 7 - protein, 16 aa, synthetic construct
  REGION 1..16: note = Synthetic construct
TMIGGSSTFYADSVNG

SEQ ID NO: 8 - protein, 17 aa, synthetic construct
  REGION 1..17: note = Synthetic construct
DVTGRSGTSIWNKRDDY

SEQ ID NO: 9 - protein, 125 aa, synthetic construct
  REGION 1..125: note = Synthetic construct
QVQLEESGGGLVQPGGSLRLSCVASGSIFSINAMGWHRQAPGSQRELVATMIGGSSTFYADSVNGRFTISRDNAKNTVYLQMNSLKLEDTAVYYCYADVTGRSGTSIWNKRDDYWGQGTLVTVSS

SEQ ID NO: 10 - protein, 16 aa, synthetic construct
  REGION 1..16: note = Synthetic construct
TMIGGSSTFYAESVQG

SEQ ID NO: 11 - protein, 125 aa, synthetic construct
  REGION 1..125: note = Synthetic construct
EVQLLESGGGLVQPGGSLRLSCAASGSIFSINAMGWHRQAPGKQRELVATMIGGSSTFYAESVQGRFTISRDNSKNTVYLQMNSLRAEDTAVYYCYADVTGRSGTSIWNKRDDYWGQGTQVTVSS

SEQ ID NO: 12 - protein, 125 aa, synthetic construct
  REGION 1..125: note = Synthetic construct
DVQLVESGGGLVQPGGSLRLSCAASGRTFSSYSMGWFRQAPGKEREFVVAISKGGYKYDAVSLEGRFTISRDNAKNTVYLQINSLRPEDTAVYYCASSRAYGSSRLRLADTYEYWGQGTLVTVSS

SEQ ID NO: 13 - protein, 453 aa, synthetic construct
  REGION 1..453: note = Synthetic construct
EVQLVESGGGLVQPGGSLRLSCAASGYDFTHYGMNWVRQAPGKGLEWVGWINTYTGEPTYAADFKRRFTFSLDTSKSTAYLQMNSLRAEDTAVYYCAKYPYYYGTSHWYFDVWGQGTLVTVSSASTKGPSVFPLAPSSKSTSGGTAALGCLVKDYFPEPVTVSWNSGALTSGVHTFPAVLQSSGLYSLSSVVTVPSSSLGTQTYICNVNHKPSNTKVDKKVEPKSCDKTHTCPPCPAPEAAGGPSVFLFPPKPKDTLMASRTPEVTCVVVDVSHEDPEVKFNWYVDGVEVHNAKTKPREEQYNSTYRVVSVLTVLAQDWLNGKEYKCKVSNKALGAPIEKTISKAKGQPREPQVYTLPPCRDELTKNQVSLWCLVKGFYPSDIAVEWESNGQPENNYKTTPPVLDSDGSFFLYSKLTVDKSRWQQGNVFSCSVMHEALHNAYTQKSLSLSPGK

SEQ ID NO: 14 - protein, 463 aa, synthetic construct
  REGION 1..463: note = Synthetic construct
QVQLVQSGAEVKKPGASVKVSCKASGYTFTGYYMHWVRQAPGQGLEWMGWINPNSGGTNYAQKFQGRVTMTRDTSISTAYMELSRLRSDDTAVYYCARSPNPYYYDSSGYYYPGAFDIWGQGTMVTVSSASVAAPSVFIFPPSDEQLKSGTASVVCLLNNFYPREAKVQWKVDNALQSGNSQESVTEQDSKDSTYSLSSTLTLSKADYEKHKVYACEVTHQGLSSPVTKSFNRGECDKTHTCPPCPAPEAAGGPSVFLFPPKPKDTLMASRTPEVTCVVVDVSHEDPEVKFNWYVDGVEVHNAKTKPREEQYNSTYRVVSVLTVLAQDWLNGKEYKCKVSNKALGAPIEKTISKAKGQPREPQVCTLPPSRDELTKNQVSLSCAVKGFYPSDIAVEWESNGQPENNYKTTPPVLDSDGSFFLVSKLTVDKSRWQQGNVFSCSVMHEALHNAYTQKSLSLSPGK

SEQ ID NO: 15 - protein, 387 aa, synthetic construct
  REGION 1..387: note = Synthetic construct
DVQLVESGGGLVQPGGSLRLSCAASGRTFSSYSMGWFRQAPGKEREFVVAISKGGYKYDAVSLEGRFTISRDNAKNTVYLQINSLRPEDTAVYYCASSRAYGSSRLRLADTYEYWGQGTLVTVSSGGGGSGGGSEVQLVESGGGLVQPGNSLRLSCAASGFTFSSFGMSWVRQAPGRGLEWVSSISGSGSDTLYADSVKGRFTISRDNAKTTLYLQMNSLRPEDTAVYYCTIGGSLSRSSQGTLVTVSSGGGGSGGGSEVQLVESGGGLVQPGGSLRLSCAVSGITLDDYAIGWFRQAPGKEREGVSAIRSSGGSTYYADSVKGRFTISSDNSKNTVYLQMNSLRPEDTAVYYCAAVPAGRLRYGEQWYPIYEYDAWGQGTLVTVSS

SEQ ID NO: 16 - protein, 10 aa, synthetic construct
  REGION 1..10: note = Synthetic construct
GFALDYYAIG

SEQ ID NO: 17 - protein, 17 aa, synthetic construct
  REGION 1..17: note = Synthetic construct
CISSGDGSTYYADSVKG

SEQ ID NO: 18 - protein, 19 aa, synthetic construct
  REGION 1..19: note = Synthetic construct
DSRGDDVACEGLRRNEYDY

SEQ ID NO: 19 - protein, 128 aa, synthetic construct
  REGION 1..128: note = Synthetic construct
QVQLVESGGGLVQPGGSLRLSCAASGFALDYYAIGWFRQAPGKEREGVSCISSGDGSTYYADSVKGRFTISRDNAKNTVYLQMNSLKPEDTAVYYCATDSRGDDVACEGLRRNEYDYWGQGTQVTVSS

SEQ ID NO: 20 - protein, 17 aa, synthetic construct
  REGION 1..17: note = Synthetic construct
CISSGEGSTYYADSVKG

SEQ ID NO: 21 - protein, 128 aa, synthetic construct
  REGION 1..128: note = Synthetic construct
EVQLLESGGGLVQPGGSLRLSCAASGFALDYYAIGWFRQAPGKGLEGVSCISSGEGSTYYADSVKGRFTISRDNSKNTVYLQMNSLRAEDTAVYYCATDSRGDDVACEGLRRNEYDYWGQGTLVTVSS

SEQ ID NO: 22 - protein, 398 aa, synthetic construct
  REGION 1..398: note = Synthetic construct
EVQLLESGGGLVQPGGSLRLSCAASGSIFSINAMGWHRQAPGKQRELVATMIGGSSTFYAESVQGRFTISRDNSKNTVYLQMNSLRAEDTAVYYCYADVTGRSGTSIWNKRDDYWGQGTQVTVSSGGGGSGGGGSEVQLLESGGGLVQPGGSLRLSCAASGSIFSINAMGWHRQAPGKQRELVATMIGGSSTFYAESVQGRFTISRDNSKNTVYLQMNSLRAEDTAVYYCYADVTGRSGTSIWNKRDDYWGQGTQVTVSSGGGGSGGGGSEVQLLESGGGLVQPGGSLRLSCAASGFALDYYAIGWFRQAPGKGLEGVSCISSGEGSTYYADSVKGRFTISRDNSKNTVYLQMNSLRAEDTAVYYCATDSRGDDVACEGLRRNEYDYWGQGTLVTVSS

SEQ ID NO: 23 - protein, 5 aa, synthetic construct
  REGION 1..5: note = Synthetic construct
  REPEAT 1..5: note = repeat 1 to 4 times
GGGGS

SEQ ID NO: 24 - protein, 574 aa, synthetic construct
  REGION 1..574: note = Synthetic construct
SDTGRPFVEMYSEIPEIIHMTEGRELVIPCRVTSPNITVTLKKFPLDTLIPDGKRIIWDSRKGFIISNATYKEIGLLTCEATVNGHLYKTNYLTHRQTNTIIDVVLSPSHGIELSVGEKLVLNCTARTELNVGIDFNWEYPSSKHQHKKLVNRDLKTQSGSEMKKFLSTLTIDGVTRSDQGLYTCAASSGLMTKKNSTFVRVHEKDKTHTCPPCPAPELLGGPSVFLFPPKPKDTLMISRTPEVTCVVVDVSHEDPEVKFNWYVDGVEVHNAKTKPREEQYNSTYRVVSVLTVLHQDWLNGKEYKCKVSNKALPAPIEKTISKAKGQPREPQVYTLPPSRDELTKNQVSLTCLVKGFYPSDIAVEWESNGQPENNYKTTPPVLDSDGSFFLYSKLTVDKSRWQQGNVFSCSVMHEALHNHYTQKSLSLSPGGGGGSGGGGSGGGGSEVQLLESGGGLVQPGGSLRLSCAASGFALDYYAIGWFRQAPGKGLEGVSCISSGEGSTYYADSVKGRFTISRDNSKNTVYLQMNSLRAEDTAVYYCATDSRGDDVACEGLRRNEYDYWGQGTLVTVSS

SEQ ID NO: 25 - protein, 431 aa, synthetic construct
  REGION 1..431: note = Synthetic construct
SDTGRPFVEMYSEIPEIIHMTEGRELVIPCRVTSPNITVTLKKFPLDTLIPDGKRIIWDSRKGFIISNATYKEIGLLTCEATVNGHLYKTNYLTHRQTNTIIDVVLSPSHGIELSVGEKLVLNCTARTELNVGIDFNWEYPSSKHQHKKLVNRDLKTQSGSEMKKFLSTLTIDGVTRSDQGLYTCAASSGLMTKKNSTFVRVHEKDKTHTCPPCPAPELLGGPSVFLFPPKPKDTLMISRTPEVTCVVVDVSHEDPEVKFNWYVDGVEVHNAKTKPREEQYNSTYRVVSVLTVLHQDWLNGKEYKCKVSNKALPAPIEKTISKAKGQPREPQVYTLPPSRDELTKNQVSLTCLVKGFYPSDIAVEWESNGQPENNYKTTPPVLDSDGSFFLYSKLTVDKSRWQQGNVFSCSVMHEALHNHYTQKSLSLSPG

SEQ ID NO: 26 - protein, 205 aa, synthetic construct
  REGION 1..205: note = Synthetic construct
SDTGRPFVEMYSEIPEIIHMTEGRELVIPCRVTSPNITVTLKKFPLDTLIPDGKRIIWDSRKGFIISNATYKEIGLLTCEATVNGHLYKTNYLTHRQTNTIIDVVLSPSHGIELSVGEKLVLNCTARTELNVGIDFNWEYPSSKHQHKKLVNRDLKTQSGSEMKKFLSTLTIDGVTRSDQGLYTCAASSGLMTKKNSTFVRVHEK

SEQ ID NO: 27 - protein, 226 aa, synthetic construct
  REGION 1..226: note = Synthetic construct
DKTHTCPPCPAPELLGGPSVFLFPPKPKDTLMISRTPEVTCVVVDVSHEDPEVKFNWYVDGVEVHNAKTKPREEQYNSTYRVVSVLTVLHQDWLNGKEYKCKVSNKALPAPIEKTISKAKGQPREPQVYTLPPSRDELTKNQVSLTCLVKGFYPSDIAVEWESNGQPENNYKTTPPVLDSDGSFFLYSKLTVDKSRWQQGNVFSCSVMHEALHNHYTQKSLSLSPG

SEQ ID NO: 28 - protein, 393 aa, synthetic construct
  REGION 1..393: note = Synthetic construct
DIQLTQSPSSLSASVGDRVTITCSASQDISNYLNWYQQKPGKAPKVLIYFTSSLHSGVPSRFSGSGSGTDFTLTISSLQPEDFATYYCQQYSTVPWTFGCGTKVEIKGGGGSGGGGSGGGGSGGGGSEVQLVESGGGLVQPGGSLRLSCAASGYDFTHYGMNWVRQAPGKCLEWVGWINTYTGEPTYAADFKRRFTFSLDTSKSTAYLQMNSLRAEDTAVYYCAKYPYYYGTSHWYFDVWGQGTLVTVSSGGGGSGGGGSGGGGSEVQLLESGGGLVQPGGSLRLSCAASGFALDYYAIGWFRQAPGKGLEGVSCISSGEGSTYYADSVKGRFTISRDNSKNTVYLQMNSLRAEDTAVYYCATDSRGDDVACEGLRRNEYDYWGQGTLVTVSS

SEQ ID NO: 29 - protein, 250 aa, synthetic construct
  REGION 1..250: note = Synthetic construct
DIQLTQSPSSLSASVGDRVTITCSASQDISNYLNWYQQKPGKAPKVLIYFTSSLHSGVPSRFSGSGSGTDFTLTISSLQPEDFATYYCQQYSTVPWTFGCGTKVEIKGGGGSGGGGSGGGGSGGGGSEVQLVESGGGLVQPGGSLRLSCAASGYDFTHYGMNWVRQAPGKCLEWVGWINTYTGEPTYAADFKRRFTFSLDTSKSTAYLQMNSLRAEDTAVYYCAKYPYYYGTSHWYFDVWGQGTLVTVSS

SEQ ID NO: 30 - protein, 107 aa, synthetic construct
  REGION 1..107: note = Synthetic construct
DIQLTQSPSSLSASVGDRVTITCSASQDISNYLNWYQQKPGKAPKVLIYFTSSLHSGVPSRFSGSGSGTDFTLTISSLQPEDFATYYCQQYSTVPWTFGCGTKVEIK

SEQ ID NO: 31 - protein, 8 aa, synthetic construct
  REGION 1..8: note = Synthetic construct
QDISNYLN

SEQ ID NO: 32 - protein, 7 aa, synthetic construct
  REGION 1..7: note = Synthetic construct
FTSSLHS

SEQ ID NO: 33 - protein, 9 aa, synthetic construct
  REGION 1..9: note = Synthetic construct
QQYSTVPWT

SEQ ID NO: 34 - protein, 123 aa, synthetic construct
  REGION 1..123: note = Synthetic construct
EVQLVESGGGLVQPGGSLRLSCAASGYDFTHYGMNWVRQAPGKCLEWVGWINTYTGEPTYAADFKRRFTFSLDTSKSTAYLQMNSLRAEDTAVYYCAKYPYYYGTSHWYFDVWGQGTLVTVSS

SEQ ID NO: 35 - protein, 7 aa, synthetic construct
  REGION 1..7: note = Synthetic construct
GYDFTHY

SEQ ID NO: 36 - protein, 6 aa, synthetic construct
  REGION 1..6: note = Synthetic construct
NTYTGE

SEQ ID NO: 37 - protein, 14 aa, synthetic construct
  REGION 1..14: note = Synthetic construct
YPYYYGTSHWYFDV

SEQ ID NO: 38 - protein, 449 aa, synthetic construct
  REGION 1..449: note = Synthetic construct
EVRLLESGGGLVQPGGSLRLSCAASGFTFSNYAMGWVRQAPGKGLEWVSAISGSGGSTYYADSVKGRFTTSRDDSKNALYLQMNSLRAEDTAVYYCARGGPGWYAADVWGQGTTVTVSSASTKGPSVFPLAPSSKSTSGGTAALGCLVKDYFPEPVTVSWNSGALTSGVHTFPAVLQSSGLYSLSSVVTVPSSSLGTQTYICNVNHKPSNTKVDKKAEPKSCDKTHTCPPCPAPELLGGPSVFLFPPKPKDTLMISRTPEVTCVVVDVSHEDPEVKFNWYVDGVEVHNAKTKPREEQYNSTYRVVSVLTVLHQDWLNGKEYKCKVSNKALPAPIEKTISKAKGQPREPQVYTLPPSRDELTKNQVSLTCLVKGFYPSDIAVEWESNGQPENNYKTTPPVLDSDGSFFLYSKLTVDKSRWQQGNVFSCSVMHEALHNHYTQKSLSLSPGK

SEQ ID NO: 39 - protein, 125 aa, synthetic construct; identical to SEQ ID NO: 12
  REGION 1..125: note = Synthetic construct

SEQ ID NO: 40 - protein, 214 aa, synthetic construct
  REGION 1..214: note = Synthetic construct
DIQLTQSPSSLSASVGDRVTITCSASQDISNYLNWYQQKPGKAPKVLIYFTSSLHSGVPSRFSGSGSGTDFTLTISSLQPEDFATYYCQQYSTVPWTFGQGTKVEIKRTVAAPSVFIFPPSDEQLKSGTASVVCLLNNFYPREAKVQWKVDNALQSGNSQESVTEQDSKDSTYSLSSTLTLSKADYEKHKVYACEVTHQGLSSPVTKSFNRGEC

SEQ ID NO: 41 - protein, 213 aa, synthetic construct
  REGION 1..213: note = Synthetic construct
SYVLTQPPSVSVAPGQTARITCGGNNIGSKSVHWYQQKPGQAPVLVVYDDSDRPSGIPERFSGSNSGNTATLTISRVEAGDEADYYCQVWDSSSDHWVFGGGTKLTVLSSASTKGPSVFPLAPSSKSTSGGTAALGCLVKDYFPEPVTVSWNSGALTSGVHTFPAVLQSSGLYSLSSVVTVPSSSLGTQTYICNVNHKPSNTKVDKKVEPKSC

SEQ ID NO: 42 - protein, 214 aa, synthetic construct
  REGION 1..214: note = Synthetic construct
DIQMTQSPSSLSASVGDRVTITCRASQSISSYLNWYQQKPGKAPKLLIYAASSLQSGVPSRFSGSGSGTDFTLTISSLQPEDFATYYCQQADLPAFAFGGGTKVEIKRTVAAPSVFIFPPSDEQLKSGTASVVCLLNNFYPREAKVQWKVDNALQSGNSQESVTEQDSKDSTYSLSSTLTLSKADYEKHKVYACEVTHQGLSSPVTKSFNRGEC

SEQ ID NO: 43 - skipped

SEQ ID NO: 44 - protein, 5 aa, artificial sequence
  REPEAT 1..5: note = This sequence may encompass 1-n repeating units, wherein n is an integer of at least 1 (and preferably 2, 3, 4, 5, 6, 7, 8, 9, 10)
GSGGS

SEQ ID NO: 45 - protein, 5 aa, artificial sequence
  REPEAT 1..5: note = This sequence may encompass 1-n repeating units, wherein n is an integer of at least 1 (and preferably 2, 3, 4, 5, 6, 7, 8, 9, 10)
GGGGS

SEQ ID NO: 46 - skipped

SEQ ID NO: 47 - protein, 6 aa, artificial sequence
  REPEAT 1..5: note = This sequence may encompass 1-n repeating units, wherein n is an integer of at least 1 (and preferably 2, 3, 4, 5, 6, 7, 8, 9, 10)
GGGGSG

SEQ ID NO: 48 - protein, 5 aa, artificial sequence
  REPEAT 1..5: note = This sequence may encompass 1-n repeating units, wherein n is an integer of 1, 2, 3 or 4
GGGGS